European Patent Specification EP 3 655 112 B1, published September 3, 2025. Title: USE OF A BACTERIAL EXTRACT FOR A COSMETIC OR DERMATOLOGICAL TREATMENT, IN PARTICULAR A MOISTURIZING TREATMENT. Applicant: SEDERMA. The sequence listing filed with the application follows.

SEQUENCE LISTING (25 sequences)

SEQ ID NO: 1 - protein, 4 aa, artificial sequence
  synthetic peptide
RSRK

SEQ ID NO: 2 - protein, 4 aa, artificial sequence
  synthetic peptide
GQPR

SEQ ID NO: 3 - protein, 4 aa, artificial sequence
  synthetic peptide
KTFK

SEQ ID NO: 4 - protein, 4 aa, Artificial sequence
  Synthetic peptide
KTAK

SEQ ID NO: 5 - protein, 4 aa, Artificial sequence
  Synthetic peptide
KAYK

SEQ ID NO: 6 - protein, 4 aa, Artificial sequence
  Synthetic peptide
KFYK

SEQ ID NO: 7 - protein, 5 aa, artificial sequence
  synthetic peptide
KTTKS

SEQ ID NO: 8 - protein, 6 aa, artificial sequence
  Synthetic peptide
GKTTKS

SEQ ID NO: 9 - protein, 6 aa, artificial sequence
  synthetic peptide
VGVAPG

SEQ ID NO: 10 - protein, 4 aa, artificial sequence
  synthetic peptide
  MOD_RES (1)..(1): amidation by a Palmitoyl chain on the N terminal end
GQPR

SEQ ID NO: 11 - protein, 4 aa, artificial sequence
  synthetic peptide
  MOD_RES (1)..(1): amidation by a Palmitoyl chain on the N terminal end
KTFK

SEQ ID NO: 12 - protein, 4 aa, artificial sequence
  synthetic peptide
  MOD_RES (1)..(1): amidation by a Elaidoyl or Palmitoyl chain on the N terminal end
KTFK

SEQ ID NO: 13 - protein, 4 aa, Artificial sequence
  Synthetic peptide
  MOD_RES (1)..(1): amidation by a Elaidoyl chain on the N terminal end
KTAK

SEQ ID NO: 14 - protein, 4 aa, Artificial sequence
  Synthetic peptide
  MOD_RES (1)..(1): amidation by a Elaidoyl chain on the N terminal end
KAYK

SEQ ID NO: 15 - protein, 4 aa, Artificial sequence
  Synthetic peptide
  MOD_RES (1)..(1): amidation by a Elaidoyl chain on the N terminal end
KFYK

SEQ ID NO: 16 - protein, 5 aa, artificial sequence
  synthetic peptide
  MOD_RES (1)..(1): amidation by a Palmitoyl chain on the N terminal end
KTTKS

SEQ ID NO: 17 - protein, 5 aa, artificial sequence
  synthetic peptide
  MOD_RES (1)..(1): amidation by a Palmitoyl chain on the N terminal end
  MISC_FEATURE (5)..(5): Xaa being either a Proline P or a Leucine L.
YGGFX

SEQ ID NO: 18 - protein, 6 aa, artificial sequence
  synthetic peptide
  MOD_RES (1)..(1): amidation by a Palmitoyl chain on the N terminal end
VGVAPG

SEQ ID NO: 19 - protein, 6 aa, artificial sequence
  synthetic peptide
  MOD_RES (1)..(1): amidation by a Palmitoyl chain on the N terminal end
GKTTKS

SEQ ID NO: 20 - protein, 6 aa, Artificial sequence
  Synthetic peptide
  MOD_RES (1)..(1): amidation by a Palmitoyl chain on the N terminal end
  MISC_FEATURE (6)..(6): Xaa being Trp, Phe, Tyr, Tic, 7-hydroxy-Tic or Tpi
HLDIIX

SEQ ID NO: 21 - protein, 6 aa, artificial sequence
  synthetic peptide
  MOD_RES (1)..(1): Acetylation on the N-terminal end
EEMQRR

SEQ ID NO: 22 - protein, 5 aa, artificial sequence
  synthetic peptide
YAGFL

SEQ ID NO: 23 - protein, 4 aa, artificial sequence
  synthetic peptide
AHSH

SEQ ID NO: 24 - protein, 6 aa, artificial sequence
  synthetic peptide
SIKVAV

SEQ ID NO: 25 - protein, 6 aa, artificial sequence
  synthetic peptide
GPQGPQ